European Patent Specification EP 3 808 369 B1, published March 26, 2025. Title: USE OF IL-22 DIMER IN MANUFACTURE OF A MEDICAMENT FOR INTRAVENOUS ADMINISTRATION. Applicant: Generon (Shanghai) Corporation Ltd. The sequence listing filed with the application follows.

SEQUENCE LISTING (10 sequences)

SEQ ID NO: 1 - protein, 16 aa, Artificial sequence
  MISC_FEATURE: short peptide
GSGGGSGGGGSGGGGS

SEQ ID NO: 2 - protein, 223 aa, Artificial sequence
  MISC_FEATURE: IgG2 Fc
VECPPCPAPPVAGPSVFLFPPKPKDTLMISRTPEVTCVVVDVSHEDPEVQFNWYVDGVEVHNAKTKPREEQFNSTFRVVSVLTVVHQDWLNGKEYKCKVSNKGLPASIEKTISKTKGQPREPQVYTLPPSREEMTKNQVSLTCLVKGFYPSDIAVEWESNGQPENNYKTTPPMLDSDGSFFLYSKLTVDKSRWQQGNVFSCSVMHEALHNHYTQKSLSLSPGK

SEQ ID NO: 3 - protein, 146 aa, Artificial sequence
  MISC_FEATURE: IL-22
APISSHCRLDKSNFQQPYITNRTFMLAKEASLADNNTDVRLIGEKLFHGVSMSERCYLMKQVLNFTLEEVLFPQSDRFQPYMQEVVPFLARLSNRLSTCHIEGDDLHIQRNVQKLKDTVKKLGESGEIKAIGELDLLFMSLRNACI

SEQ ID NO: 4 - protein, 385 aa, Artificial sequence
  MISC_FEATURE: IL-22－linker－IgG2 Fc
APISSHCRLDKSNFQQPYITNRTFMLAKEASLADNNTDVRLIGEKLFHGVSMSERCYLMKQVLNFTLEEVLFPQSDRFQPYMQEVVPFLARLSNRLSTCHIEGDDLHIQRNVQKLKDTVKKLGESGEIKAIGELDLLFMSLRNACIGSGGGSGGGGSGGGGSVECPPCPAPPVAGPSVFLFPPKPKDTLMISRTPEVTCVVVDVSHEDPEVQFNWYVDGVEVHNAKTKPREEQFNSTFRVVSVLTVVHQDWLNGKEYKCKVSNKGLPASIEKTISKTKGQPREPQVYTLPPSREEMTKNQVSLTCLVKGFYPSDIAVEWESNGQPENNYKTTPPMLDSDGSFFLYSKLTVDKSRWQQGNVFSCSVMHEALHNHYTQKSLSLSPGK

SEQ ID NO: 5 - protein, 308 aa, Artificial sequence
  MISC_FEATURE: IL-22－linker－IL-22
APISSHCRLDKSNFQQPYITNRTFMLAKEASLADNNTDVRLIGEKLFHGVSMSERCYLMKQVLNFTLEEVLFPQSDRFQPYMQEVVPFLARLSNRLSTCHIEGDDLHIQRNVQKLKDTVKKLGESGEIKAIGELDLLFMSLRNACIGSGGGSGGGGSGGGGSAPISSHCRLDKSNFQQPYITNRTFMLAKEASLADNNTDVRLIGEKLFHGVSMSERCYLMKQVLNFTLEEVLFPQSDRFQPYMQEVVPFLARLSNRLSTCHIEGDDLHIQRNVQKLKDTVKKLGESGEIKAIGELDLLFMSLRNACI

SEQ ID NO: 6 - protein, 375 aa, Artificial sequence
  MISC_FEATURE: IL-22-linker-IgG2 Fc
APISSHCRLDKSNFQQPYITNRTFMLAKEASLADNNTDVRLIGEKLFHGVSMSERCYLMKQVLNFTLEEVLFPQSDRFQPYMQEVVPFLARLSNRLSTCHIEGDDLHIQRNVQKLKDTVKKLGESGEIKAIGELDLLFMSLRNACIASTKGPVECPPCPAPPVAGPSVFLFPPKPKDTLMISRTPEVTCVVVDVSHEDPEVQFNWYVDGVEVHNAKTKPREEQFNSTFRVVSVLTVVHQDWLNGKEYKCKVSNKGLPASIEKTISKTKGQPREPQVYTLPPSREEMTKNQVSLTCLVKGFYPSDIAVEWESNGQPENNYKTTPPMLDSDGSFFLYSKLTVDKSRWQQGNVFSCSVMHEALHNHYTQKSLSLSPGK

SEQ ID NO: 7 - protein, 385 aa, Artificial sequence [sequence omitted]

SEQ ID NO: 8 - protein, 375 aa, Artificial sequence
  MISC_FEATURE: IgG2 Fc-linker- IL-22
VECPPCPAPPVAGPSVFLFPPKPKDTLMISRTPEVTCVVVDVSHEDPEVQFNWYVDGVEVHNAKTKPREEQFNSTFRVVSVLTVVHQDWLNGKEYKCKVSNKGLPASIEKTISKTKGQPREPQVYTLPPSREEMTKNQVSLTCLVKGFYPSDIAVEWESNGQPENNYKTTPPMLDSDGSFFLYSKLTVDKSRWQQGNVFSCSVMHEALHNHYTQKSLSLSPGKASTKGPAPISSHCRLDKSNFQQPYITNRTFMLAKEASLADNNTDVRLIGEKLFHGVSMSERCYLMKQVLNFTLEEVLFPQSDRFQPYMQEVVPFLARLSNRLSTCHIEGDDLHIQRNVQKLKDTVKKLGESGEIKAIGELDLLFMSLRNACI

SEQ ID NO: 9 - protein, 228 aa, homo sapiens
ERKCCVECPPCPAPPVAGPSVFLFPPKPKDTLMISRTPEVTCVVVDVSHEDPEVQFNWYVDGVEVHNAKTKPREEQFNSTFRVVSVLTVVHQDWLNGKEYKCKVSNKGLPAPIEKTISKTKGQPREPQVYTLPPSREEMTKNQVSLTCLVKGFYPSDISVEWESNGQPENNYKTTPPMLDSDGSFFLYSKLTVDKSRWQQGNVFSCSVMHEALHNHYTQKSLSLSPGK

SEQ ID NO: 10 - protein, 6 aa, Artificial sequence
  MISC_FEATURE: short peptide
ASTKGP